European Patent Application EP 4 335 922 A1, published March 13, 2024. Title: WASCH- UND REINIGUNGSMITTEL ENTHALTEND TANNASE I. Applicant: Henkel AG & Co. KGaA. The sequence listing filed with the application follows.

SEQUENCE LISTING (1 sequence)

SEQ ID NO: 1 - protein, 511 aa, Streptomyces ipomoeae
MKRRSVVMGLTAAAAVPSVGLASGARAADGTSATAGSAGTTAASVAGSSSLVFDPAAHTEQTVAITDTTGTAHEVVYRFYKVASYVANPVDAAYQSLNVCEPVKIDGVAVDAGRAPILLANAVGGYMPSSVAGKTGITATGMGGATSRQALALAAGYVVVEPGARGRTLVDASGVHYGVAPAAIVDLKAAVRYLKFNKGRVPGNVNRIVSSGVSAGGALSSLLGASGDSSLYEPYLEAIGAADASDAIFATGAWCPITDLEHADMAYEWCWGGNPLAGGSQADQTLSNELRTAYGDHVASLGLRARGYGRLTARNLDDYLLKTFMEPSATKYLAALSETDRSAYLAANPFITWSGGRASFTWADFVTHVGTRRKNVPSFDTFDMASPENNLFGVGTTRARHFTLWSLRKQQGDSARLDEDIPEKLALMNPMHHLADKPNAHRSKHWWIRLGTKDTDTSHTVVGNLHARLVQLGDDVNTSYYWDAGHGADQDPGDFVTWIGEVSGYRSKVRK